European Patent Application EP 4 163 383 A1, published April 12, 2023. Title: MICROBIAL PRODUCTION OF FATTY AMINES. Applicant: Genomatica, Inc. Application EP. The sequence listing filed with the application follows.

SEQUENCE LISTING (2 sequences)

SEQ ID NO: 1 - DNA, 43 bp, synthetic construct
  source 1..43: mol_type = other DNA
aggaggaataacatatgaacaggttaccttcgagcgcatcggc

SEQ ID NO: 2 - DNA, 47 bp, synthetic construct
  source 1..47: mol_type = other DNA
cccaagcttcgaattcttacgcttcttcgacacttactcgcatggcc